European Patent Specification EP 3 436 595 B1, published February 28, 2024. Title: OPTIMIZED MICROBIAL CELLS FOR PRODUCTION OF MELATONIN AND OTHER COMPOUNDS. Applicant: Danmarks Tekniske Universitet. The sequence listing filed with the application follows.

SEQUENCE LISTING (64 sequences)

SEQ ID NO: 1 - protein, 444 aa, Oryctolagus cuniculus
MIEDNKENKDHSLERGRATLIFSLKNEVGGLIKALKIFQEKHVNLLHIESRKSKRRNSEFEIFVDCDTNREQLNDIFHLLKSHTNVLSVTPPDNFTMKEEGMESVPWFPKKISDLDHCANRVLMYGSELDADHPGFKDNVYRKRRKYFADLAMSYKYGDPIPKVEFTEEEIKTWGTVFRELNKLYPTHACREYLKNLPLLSKYCGYREDNIPQLEDISNFLKERTGFSIRPVAGYLSPRDFLSGLAFRVFHCTQYVRHSSDPFYTPEPDTCHELLGHVPLLAEPSFAQFSQEIGLASLGASEEAVQKLATCYFFTVEFGLCKQDGQLRVFGAGLLSSISELKHVLSGHAKVKPFDPKITYKQECLITTFQDVYFVSESFEDAKEKMREFTKTIKRPFGVKYNPYTRSIQILKDAKSITNAMNELRHDLDVVSDALGKVSRQLSV

SEQ ID NO: 2 - protein, 444 aa, Homo sapiens
MIEDNKENKDHSLERGRASLIFSLKNEVGGLIKALKIFQEKHVNLLHIESRKSKRRNSEFEIFVDCDINREQLNDIFHLLKSHTNVLSVNLPDNFTLKEDGMETVPWFPKKISDLDHCANRVLMYGSELDADHPGFKDNVYRKRRKYFADLAMNYKHGDPIPKVEFTEEEIKTWGTVFQELNKLYPTHACREYLKNLPLLSKYCGYREDNIPQLEDVSNFLKERTGFSIRPVAGYLSPRDFLSGLAFRVFHCTQYVRHSSDPFYTPEPDTCHELLGHVPLLAEPSFAQFSQEIGLASLGASEEAVQKLATCYFFTVEFGLCKQDGQLRVFGAGLLSSISELKHALSGHAKVKPFDPKITCKQECLITTFQDVYFVSESFEDAKEKMREFTKTIKRPFGVKYNPYTRSIQILKDTKSITSAMNELQHDLDVVSDALAKVSRKPSI

SEQ ID NO: 3 - protein, 490 aa, Homo sapiens
MQPAMMMFSSKYWARRGFSLDSAVPEEHQLLGSSTLNKPNSGKNDDKGNKGSSKREAATESGKTAVVFSLKNEVGGLVKALRLFQEKRVNMVHIESRKSRRRSSEVEIFVDCECGKTEFNELIQLLKFQTTIVTLNPPENIWTEEEELEDVPWFPRKISELDKCSHRVLMYGSELDADHPGFKDNVYRQRRKYFVDVAMGYKYGQPIPRVEYTEEETKTWGVVFRELSKLYPTHACREYLKNFPLLTKYCGYREDNVPQLEDVSMFLKERSGFTVRPVAGYLSPRDFLAGLAYRVFHCTQYIRHGSDPLYTPEPDTCHELLGHVPLLADPKFAQFSQEIGLASLGASDEDVQKLATCYFFTIEFGLCKQEGQLRAYGAGLLSSIGELKHALSDKACVKAFDPKTTCLQECLITTFQEAYFVSESFEEAKEKMRDFAKSITRPFSVYFNPYTQSIEILKDTRSIENVVQDLRSDLNTVCDALNKMNQYLGI

SEQ ID NO: 4 - protein, 502 aa, Bos taurus
MQPAMMMFSSKYWARRGLSLDSAVPEEHQLLTSLTLNKTNSGKNDDKKGNKGSSKNDTATESGKTAVVFSLKNEVGGLVKALKLFQEKHVNMIHIESRKSRRRSSEVEIFVDCECGKTEFNELIQSLKFQTTIVTLNPPENIWTEEEGKLTCVAKGKELEDVPWFPRKISELDRCSHRVLMYGSELDADHPGFKDNVYRQRRKYFVDVAMGYKYGQPIPRVEYTEEETKTWGVVFRELSKLYPTHACREYLKNFPLLTKHCGYREDNVPQLEDVAAFLKERSGFTVRPVAGYLSPRDFLAGLAYRVFHCTQYVRHGSDPLYTPEPDVTLSLLSHVPLIFDDQFPTSFSNEVGRAVILASWGDKQENNQCYFFTIEFGLCKQEGQLRAYGAGLLSSIGELKHALSDKACVKAFDPKTTCLQECLITTFQEAYFVSESFEEAKEKMRDFAKSITRPFSVYFNPYTQSIEILKDTRSIENVVQDLRSDLNTVCDALNKMNQYLGI

SEQ ID NO: 5 - protein, 497 aa, Sus scrofa
MQPAMMMFSSKYWARRGLSLDSAVPEEHQLLGSLTVSTFLKLNKSNSGKNDDKKGNKGSGKSDTATESGKTAVVFSLKNEVGGLVKALKLFQEKHVNMVHIESRKSRRRSSEVEIFVDCECGKTEFNELIQSLKFQTTIVTLNPPENIWTEEEELEDVPWFPRKISELDKCSHRVLMYGSELDADHPGFKDNVYRQRRKYFVDLAMGYKYGQPIPRVEYTEEETKTWGIVFRELSKLYPTHACREYLKNFPLLTKYCGYREDNVPQLEDVSVFLKERSGFTVRPVAGYLSPRDFLAGLAYRVFHCTQYVRHGSDPLYTPEPDTCHELLGHVPLLADPKFAQFSQEIGLASLGASDEDVQKLATCYFFTIEFGLCKQEGQLRAYGAGLLSSIGELKHALSDKACVKAFDPKTTCLQECLITTFQEAYFVSESFEEAKEKMRDFAKSITRPFSVYFNPYTQSIEILKDTRSIENVVQDLRSDLNTVCDALNKMNQYLGI

SEQ ID NO: 6 - protein, 445 aa, Gallus gallus
MIEDNKENKDHAPERGRTAIIFSLKNEVGGLVKALKLFQEKHVNLVHIESRKSKRRNSEFEIFVDCDSNREQLNEIFQLLKSHVSIVSMNPTEHFNVQEDGDMENIPWYPKKISDLDKCANRVLMYGSDLDADHPGFKDNVYRKRRKYFADLAMNYKHGDPIPEIEFTEEEIKTWGTVYRELNKLYPTHACREYLKNLPLLTKYCGYREDNIPQLEDVSRFLKERTGFTIRPVAGYLSPRDFLAGLAFRVFHCTQYVRHSSDPLYTPEPDTCHELLGHVPLLAEPSFAQFSQEIGLASLGASDEAVQKLATCYFFTVEFGLCKQEGQLRVYGAGLLSSISELKHSLSGSAKVKPFDPKVTCKQECLITTFQEVYFVSESFEEAKEKMREFAKTIKRPFGVKYNPYTQSVQILKDTKSIASVVNELRHELDIVSDALSKMGKQLEV

SEQ ID NO: 7 - protein, 447 aa, Mus musculus
MIEDNKENKENKDHSSERGRVTLIFSLENEVGGLIKVLKIFQENHVSLLHIESRKSKQRNSEFEIFVDCDISREQLNDIFPLLKSHATVLSVDSPDQLTAKEDVMETVPWFPKKISDLDFCANRVLLYGSELDADHPGFKDNVYRRRRKYFAELAMNYKHGDPIPKIEFTEEEIKTWGTIFRELNKLYPTHACREYLRNLPLLSKYCGYREDNIPQLEDVSNFLKERTGFSIRPVAGYLSPRDFLSGLAFRVFHCTQYVRHSSDPLYTPEPDTCHELLGHVPLLAEPSFAQFSQEIGLASLGASEETVQKLATCYFFTVEFGLCKQDGQLRVFGAGLLSSISELKHALSGHAKVKPFDPKIACKQECLITSFQDVYFVSESFEDAKEKMREFAKTVKRPFGLKYNPYTQSVQVLRDTKSITSAMNELRYDLDVISDALARVTRWPSV

SEQ ID NO: 8 - protein, 491 aa, Equus caballus
MQPAMMMFSSKYWARRGFSLDSAVPEEHQLLGNLTVNKSNSGKNDDKKGNKGSSRSETAPDSGKTAVVFSLRNEVGGLVKALKLFQEKHVNMVHIESRKSRRRSSEVEIFVDCECGKTEFNELIQLLKFQTTIVTLNPPENIWTEEEELEDVPWFPRKISELDKCSHRVLMYGSELDADHPGFKDNVYRQRRKYFVDVAMSYKYGQPIPRVEYTEEETKTWGVVFRELSRLYPTHACQEYLKNFPLLTKYCGYREDNVPQLEDVSMFLKERSGFAVRPVAGYLSPRDFLAGLAYRVFHCTQYVRHSSDPLYTPEPDTCHELLGHVPLLADPKFAQFSQEIGLASLGASDEDVQKLATCYFFTIEFGLCKQEGQLRAYGAGLLSSIGELKHALSDKACVKAFDPKTTCLQECLITTFQEAYFVSESFEEAKEKMREFAKSITRPFSVHFNPYTQSVEVLKDSRSIESVVQDLRSDLNTVCDALNKMNQYLGV

SEQ ID NO: 9 - protein, 497 aa, Schistosoma mansoni
MISTESDLRRQLDENVRSEADESTKEECPYINAVQSHHQNVQEMSIIISLVKNMNDMKSIISIFTDRNINILHIESRLGRLNMKKHTEKSEFEPLELLVHVEVPCIEVERLLEELKSFSSYRIVQNPLMNLPEAKNPTLDDKVPWFPRHISDLDKVSNSVLMYGKELDADHPGFKDKEYRKRRMMFADIALNYKWGQQIPIVEYTEIEKTTWGRIYRELTRLYKTSACHEFQKNLGLLQDKAGYNEFDLPQLQVVSDFLKARTGFCLRPVAGYLSARDFLSGLAFRVFYCTQYIRHQADPFYTPEPDCCHELLGHVPMLADPKFARFSQEIGLASLGTSDEEIKKLATCYFFTIEFGLCRQDNQLKAYGAGLLSSVAELQHALSDKAVIKPFIPMKVINEECLVTTFQNGYFETSSFEDATRQMREFVRTIKRPFDVHYNPYTQSIEIIKTPKSVAKLVQDLQFELTAINESLLKMNKEIRSQQFTTNKIVTENRSS

SEQ ID NO: 10 - protein, 496 aa, Homo sapiens [sequence omitted]

SEQ ID NO: 11 - protein, 448 aa, Homo sapiens
MDDKGNKGSSKREAATESGKTAVVFSLKNEVGGLVKALRLFQEKRVNMVHIESRKSRRRSSEVEIFVDCECGKTEFNELIQLLKFQTTIVTLNPPENIWTEEEELEDVPWFPRKISELDKCSHRVLMYGSELDADHPGFKDNVYRQRRKYFVDVAMGYKYGQPIPRVEYTEEETKTWGVVFRELSKLYPTHACREYLKNFPLLTKYCGYREDNVPQLEDVSMFLKERSGFTVRPVAGYLSPRDFLAGLAYRVFHCTQYIRHGSDPLYTPEPDTCHELLGHVPLLADPKFAQFSQEIGLASLGASDEDVQKLATCYFFTIEFGLCKQEGQLRAYGAGLLSSIGELKHALSDKACVKAFDPKTTCLQECLITTFQEAYFVSESFEEAKEKMRDFAKSITRPFSVYFNPYTQSIEILKDTRSIENVVQDLRINRVHSSALTEKEGVRQPEV

SEQ ID NO: 12 - protein, 428 aa, Homo sapiens
MDDKGNKGSSKREAATESGKTAVVFSLKNEVGGLVKALRLFQEKRVNMVHIESRKSRRRSSEVEIFVDCECGKTEFNELIQLLKFQTTIVTLNPPENIWTEEEELEDVPWFPRKISELDKCSHRVLMYGSELDADHPGFKDNVYRQRRKYFVDVAMGYKYGQPIPRVEYTEEETKTWGVVFRELSKLYPTHACREYLKNFPLLTKYCGYREDNVPQLEDVSMFLKERSGFTVRPVAGYLSPRDFLAGLAYRVFHCTQYIRHGSDPLYTPEPDTCHELLGHVPLLADPKFAQFSQEIGLASLGASDEDVQKLATCYFFTIEFGLCKQEGQLRAYGAGLLSSIGELKHALSDKACVKAFDPKTTCLQECLITTFQEAYFVSESFEEAKEKMRDFAKSITRPFSVYFNPYTQSIEILKDTRSIENVVQDLR

SEQ ID NO: 13 - protein, 315 aa, Homo sapiens
MELEDVPWFPRKISELDKCSHRVLMYGSELDADHPGFKDNVYRQRRKYFVDVAMGYKYGQPIPRVEYTEEETKTWGVVFRELSKLYPTHACREYLKNFPLLTKYCGYREDNVPQLEDVSMFLKERSGFTVRPVAGYLSPRDFLAGLAYRVFHCTQYIRHGSDPLYTPEPDTCHELLGHVPLLADPKFAQFSQEIGLASLGASDEDVQKLATCYFFTIEFGLCKQEGQLRAYGAGLLSSIGELKHALSDKACVKAFDPKTTCLQECLITTFQEAYFVSESFEEAKEKMRDFAKSITRPFSVYFNPYTQSIEILKDT

SEQ ID NO: 14 - protein, 250 aa, Homo sapiens
MEKGPVRAPAEKPRGARCSNGFPERDPPRPGPSRPAEKPPRPEAKSAQPADGWKGERPRSEEDNELNLPNLAAAYSSILSSLGENPQRQGLLKTPWRAASAMQFFTKGYQETISDVLNDAIFDEDHDEMVIVKDIDMFSMCEHHLVPFVGKVHIGYLPNKQVLGLSKLARIVEIYSRRLQVQERLTKQIAVAITEALRPAGVGVVVEATHMCMVMRGVQKMNSKTVTSTMLGVFREDPKTREEFLTLIRS

SEQ ID NO: 15 - protein, 241 aa, Mus musculus
MEKPRGVRCTNGFSERELPRPGASPPAEKSRPPEAKGAQPADAWKAGRHRSEEENQVNLPKLAAAYSSILLSLGEDPQRQGLLKTPWRAATAMQYFTKGYQETISDVLNDAIFDEDHDEMVIVKDIDMFSMCEHHLVPFVGRVHIGYLPNKQVLGLSKLARIVEIYSRRLQVQERLTKQIAVAITEALQPAGVGVVIEATHMCMVMRGVQKMNSKTVTSTMLGVFREDPKTREEFLTLIRS

SEQ ID NO: 16 - protein, 222 aa, Escherichia coli
MPSLSKEAALVHEALVARGLETPLRPPVHEMDNETRKSLIAGHMTEIMQLLNLDLADDSLMETPHRIAKMYVDEIFSGLDYANFPKITLIENKMKVDEMVTVRDITLTSTCEHHFVTIDGKATVAYIPKDSVIGLSKINRIVQFFAQRPQVQERLTQQILIALQTLLGTNNVAVSIDAVHYCVKARGIRDATSATTTTSLGGLFKSSQNTRHEFLRAVRHHN

SEQ ID NO: 17 - protein, 243 aa, Saccharomyces cerevisiae
MHNIQLVQEIERHETPLNIRPTSPYTLNPPVERDGFSWPSVGTRQRAEETEEEEKERIQRISGAIKTILTELGEDVNREGLLDTPQRYAKAMLYFTKGYQTNIMDDVIKNAVFEEDHDEMVIVRDIEIYSLCEHHLVPFFGKVHIGYIPNKKVIGLSKLARLAEMYARRLQVQERLTKQIAMALSDILKPLGVAVVMEASHMCMVSRGIQKTGSSTVTSCMLGGFRAHKTREEFLTLLGRRSI

SEQ ID NO: 18 - protein, 190 aa, Bacillus subtilis
MKEVNKEQIEQAVRQILEAIGEDPNREGLLDTPKRVAKMYAEVFSGLNEDPKEHFQTIFGENHEELVLVKDIAFHSMCEHHLVPFYGKAHVAYIPRGGKVTGLSKLARAVEAVAKRPQLQERITSTIAESIVETLDPHGVMVVVEAEHMCMTMRGVRKPGAKTVTSAVRGVFKDDAAARAEVLEHIKRQD

SEQ ID NO: 19 - protein, 201 aa, Streptomyces avermitilis
MTDPVTLDGEGTIGEFDEKRAENAVRELLIAVGEDPDREGLRETPGRVARAYREIFAGLWQKPEDVLTTTFDIGHDEMVLVKDIEVLSSCEHHLVPFVGVAHVGYIPSTDGKITGLSKLARLVDVYARRPQVQERLTTQVADSLMEILEPRGVIVVVECEHMCMSMRGVRKPGAKTITSAVRGQLRDPATRNEAMSLIMAR

SEQ ID NO: 20 - protein, 222 aa, Salmonella typhi
MPSLSKEAALVHDALVARGLETPLRPPMDELDNETRKSLIAGHMTEIMQLLNLDLSDDSLMETPHRIAKMYVDEIFAGLDYANFPKITLIENKMKVDEMVTVRDITLTSTCEHHFVTIDGKATVAYIPKDSVIGLSKINRIVQFFAQRPQVQERLTQQILTALQTLLGTNNVAVSIDAVHYCVKARGIRDATSATTTTSLGGLFKSSQNTRQEFLRAVRHHP

SEQ ID NO: 21 - protein, 108 aa, Chromobacterium violaceum
MNLLELSCTPQHGQSPLADNTVKQLLSTLPDWEIVGIELRKTYRFANYHETMAFVNALAWIANQEDHHPDMSVHYNRAVVNFSTHDAGGLTLNDFICAAKTEALFRRP

SEQ ID NO: 22 - protein, 118 aa, Pseudomonas aeruginosa
MTALTQAHCEACRADAPHVSDEELPVLLRQIPDWNIEVRDGIMQLEKVYLFKNFKHALAFTNAVGEISEAEGHHPGLLTEWGKVTVTWWSHSIKGLHRNDFIMAARTDEVAKTAEGRK

SEQ ID NO: 23 - protein, 104 aa, Bacillus cereus var. anthracis
MMLRLTEEEVQEELLKLDKWVVKDEKWIERKYMFSDYLKGVEFVSEAAKLSEEHNHHPFILIQYKAVIITLSSWNAKGLTKLDFELAKQFDELFVQNEKAVIRK

SEQ ID NO: 24 - protein, 188 aa, Corynebacterium genitalium
MSDTLDALDIHEPDEAFLMATEAEVEVPSQPCALAVLVSDHKQGGAIDEGTDRLVFELLQEIGFKVDGVVYVKSKKSEIRKVIETAVVGGVDLVVTVGGTGVGPRDKAPEATRGVIDQLVPGVAQAVRASGQACGAVDACTSRGICGVSGSTVVVNLAPSRAAIRDGISTISPLVAHLISELRKYSVQ

SEQ ID NO: 25 - protein, 63 aa, Lactobacillus ruminis
MVKLFPSENARRWHRWNHEVLLLVNIQCSLKQPLWSAEGKVDKNREKCAAFVYRLVEIQDARI

SEQ ID NO: 26 - protein, 96 aa, Rhodobacteraceae bacterium
MSERLFDDTRGPLLDPLFATGWAMVEGRDAIEKHYKFKNFADAFGWMTRAAIWSEKWDHHPEWLNVYNKVHVVLTTHSVDGLSPLDVKLARKFDSL

SEQ ID NO: 27 - protein, 104 aa, Homo sapiens
MAGKAHRLSAEERDQLLPNLRAVGWNELEGRDAIFKQFHFKDFNRAFGFMTRVALQAEKLDHHPEWFNVYNKVHITLSTHECAGLSERDINLASFIEQVAVSMT

SEQ ID NO: 28 - protein, 430 aa, Acidobacterium capsulatum
SAGQAYADYLHLVQPYTNGNRHPRAWGWVRGNGTPIGAMAEMLAAAINPHLGGGDQSPTYVEERCLQWLAQVMGMPATATGILTSGGTMANLLGLAVARHAKAGFDVRAEGLAAHTPLTVYASSEAHMWAGNAMDLLGLGSSRLRSIPVDENFRIDLAALRLKIREDRAAGLQPIAVIGNAGTVNTGAVDDLEALAALCREEELWFHVDGAFGALLKLSPRHASLVRGLEQADSLAFDLHKWMYLPFEIGCVLVANGEEHRAAFASSASYLEGAKRGILATGLIFADRGLELTRGFKALKLWMALKAHGLNAFSEMIEQNMAQARYLERRVLEEPELELLAPRSMNIVCFRYRGRGAAGDELLNALNRELVLRLQESGEFVVSGTMLKGRYALRIANTNHRSRLQDFEDLVQWSLKLGCEIEAESQAART

SEQ ID NO: 29 - protein, 480 aa, Rattus norvegicus
MDSREFRRRGKEMVDYIADYLDGIEGRPVYPDVEPGYLRALIPTTAPQEPETYEDIIRDIEKIIMPGVTHWHSPYFFAYFPTASSYPAMLADMLCGAIGCIGFSWAASPACTELETVMMDWLGKMLELPEAFLAGRAGEGGGVIQGSASEATLVALLAARTKMIRQLQAASPELTQAALMEKLVAYTSDQAHSSVERAGLIGGVKIKAIPSDGNYSMRAAALREALERDKAAGLIPFFVVVTLGTTSCCSFDNLLEVGPICNQEGVWLHIDAAYAGSAFICPEFRYLLNGVEFADSFNFNPHKWLLVNFDCSAMWVKKRTDLTEAFNMDPVYLRHSHQDSGLITDYRHWQIPLGRRFRSLKMWFVFRMYGVKGLQAYIRKHVKLSHEFESLVRQDPRFEICTEVILGLVCFRLKGSNQLNETLLQRINSAKKIHLVPCRLRDKFVLRFAVCSRTVESAHVQLAWEHIRDLASSVLRAEKE

SEQ ID NO: 30 - protein, 486 aa, Sus scrofa
MNASDFRRRGKEMVDYMADYLEGIEGRQVYPDVQPGYLRPLIPATAPQEPDTFEDILQDVEKIIMPGVTHWHSPYFFAYFPTASSYPAMLADMLCGAIGCIGFSWAASPACTELETVMMDWLGKMLQLPEAFLAGEAGEGGGVIQGSASEATLVALLAARTKVVRRLQAASPGLTQGAVLEKLVAYASDQAHSSVERAGLIGGVKLKAIPSDGKFAMRASALQEALERDKAAGLIPFFVVATLGTTSCCSFDNLLEVGPICHEEDIWLHVDAAYAGSAFICPEFRHLLNGVEFADSFNFNPHKWLLVNFDCSAMWVKRRTDLTGAFKLDPVYLKHSHQGSGLITDYRHWQLPLGRRFRSLKMWFVFRMYGVKGLQAYIRKHVQLSHEFEAFVLQDPRFEVCAEVTLGLVCFRLKGSDGLNEALLERINSARKIHLVPCRLRGQFVLRFAICSRKVESGHVRLAWEHIRGLAAELLAAEEGKAEIKS

SEQ ID NO: 31 - protein, 480 aa, Homo sapiens
MNASEFRRRGKEMVDYMANYMEGIEGRQVYPDVEPGYLRPLIPAAAPQEPDTFEDIINDVEKIIMPGVTHWHSPYFFAYFPTASSYPAMLADMLCGAIGCIGFSWAASPACTELETVMMDWLGKMLELPKAFLNEKAGEGGGVIQGSASEATLVALLAARTKVIHRLQAASPELTQAAIMEKLVAYSSDQAHSSVERAGLIGGVKLKAIPSDGNFAMRASALQEALERDKAAGLIPFFMVATLGTTTCCSFDNLLEVGPICNKEDIWLHVDAAYAGSAFICPEFRHLLNGVEFADSFNFNPHKWLLVNFDCSAMWVKKRTDLTGAFRLDPTYLKHSHQDSGLITDYRHWQIPLGRRFRSLKMWFVFRMYGVKGLQAYIRKHVQLSHEFESLVRQDPRFEICVEVILGLVCFRLKGSNKVNEALLQRINSAKKIHLVPCHLRDKFVLRFAICSRTVESAHVQRAWEHIKELAADVLRAERE

SEQ ID NO: 32 - protein, 503 aa, Capsicum annuum
MGSLDSNNSTQTQSNVTKFNPLDPEEFRTQAHQMVDFIADYYKNIESYPVLSQVEPGYLRNHLPENAPYLPESLDTIMKDVEKHIIPGMTHWLSPNFFAFFPATVSSAAFLGEMLCNCFNSVGFNWLASPAMTELEMIIMDWLANMLKLPECFMFSGTGGGVIQGTTSEAILCTLIAARDRKLENIGVDNIGKLVVYGSDQTHSMYAKACKAAGIFPCNIRAISTCVENDFSLSPAVLRGIVEVDVAAGLVPLFLCATVGTTSTTAIDPISELGELANEFDIWLHVDAAYGGSACICPEFRQYLDGIERANSFSLSPHKWLLSYLDCCCMWVKEPSVLVKALSTNPEYLRNKRSEHGSVVDYKDWQIGTGRKFKSLRLWLIMRSYGVANLQSHIRSDVRMAKMFEGLVRSDPYFEVIVPRRFSLVCFRFNPDKEYEPAYTELLNKRLLDNVNSTGRVYMTHTVAGGIYMLRFAVGATFTEDRHLICAWKLIKDCADALLRNCQ

SEQ ID NO: 33 - protein, 281 aa, Drosophila caribiana
  misc_feature (79)..(79): Xaa can be any naturally occurring amino acid
MLDLPAEFLACSGGKGGGVIQGTASESTLVALLGAKAKKLQEVKAEHPEWDDHTIIGKLVGYTSAQSHSSVERAGLLGXIKLRSVPADEHNRLRGDALEKAIEKDLAEGLIPFYAVVTLGTTNSCAFDRLDECGPVANKHKVWVHVDAAYAGSAFICPEYRHHMKGIETADSFNFNPHKWMLVNFDCSAMWLKDPSWVVNAFNVDPLYLKHDMQGSAPDYRHWQIPLGRRFRALKLWFVLRLYGVENLQAHIRRHCGFAQQFADLCVADERFELAAEVNMG

SEQ ID NO: 34 - protein, 478 aa, Maricaulis maris
MHGRCKKLRLPPGMIMKLEEFGLWSRRIADWSKTYLETLRERPVRPATRPADVLNALPVTPPEDATDMAEIFADFERIVPDAMTHWQHPRFFAYFPANAAPASILAEQLVSTMAAQCMLWQTSPAATEMETRMVDWLRQALGLPDGWRGVIQDSASSATLSAVMTMRERALDWRGIRSGLAGEKAPRIYASAQTHSSVDKACWVAGIGQDNLVKIATTDDYGMDPDALRAAIRADRAAGHLPAGIVICVGGTAIGASDPVAAIIEVARAEGLYTHIDAAWAGSAMICPELRHIWEGAEGADSIVFNPHKWLGAQFDCSVQFLRDPTDQLKSLTLRPDYLETPGMDDAVNYSEWTIPLGRRFRALKLWFLIRAYGLEGLRTRIRNHIAWSNEACEAIRDLPGLEIVTEPRFSLFSFACTAGDEATADLLERINSDGRTYLTQTRHEGRYVIRLQVGQFDCTRADVMEAVAVIGELRGEG

SEQ ID NO: 35 - protein, 523 aa, Oryza sativa
MGSLDANPAAAYAAFAADVEPFRPLDADDVRSYLHKAVDFVYDYYKSVESLPVLPGVEPGYLLRLLQSAPPSSSAPFDIAMKELREAVVPGMTHWASPNFFAFFPATNSAAAIAGELIASAMNTVGFTWQAAPAATELEVLALDWLAQLLGLPASFMNRTVAGGRGTGGGVILGTTSEAMLVTLVAARDAALRRSGSNGVAGITRLTVYAADQTHSTFFKACRLAGFDPANIRSIPTGAETDYGLDPARLLEAMQADADAGLVPTYVCATVGTTSSNAVDPVGAVADVAARFAAWVHVDAAYAGSACICPEFRHHLDGVERVDSISMSPHKWLMTCLDCTCLYVRDTHRLTGSLETNPEYLKNHASDSGEVTDLKDMQVGVGRRFRGLKLWMVMRTYGAGKLQEHIRSDVAMAKTFEDLVRGDDRFEVVVPRNFALVCFRIRPRKSGAAIAAGEAEAEKANRELMERLNKTGKAYVAHTVVGGRFVLRFAVGSSLQEERHVRSAWELIKKTTTEIVADAGEDK

SEQ ID NO: 36 - protein, 470 aa, Pseudomonas putida
MTPEQFRQYGHQLIDLIADYRQTVGERPVMAQVEPGYLKAALPAQAPRQGEPFAAILDDVNQLVMPGLSHWQHPDFYGYFPSNGTLSSVLGDFLSTGLGVLGLSWQSSPALSELEETTLDWLRQLLGLSGQWSGVIQDTASTSTLVALICARERASDYALVRGGLQAQAKPLIVYVSAHAHSSVDKAALLAGFGRDNIRLIPTDERYALRPEALQVAIEQDLAAGNQPCAVVATTGTTATTALDPLRPIGEIAQAHGLWLHVDSAMAGSAMILPECRWMWDGIELADSLVVNAHKWLGVAFDCSIYYVRDPQHLIRVMSTNPSYLQSSVDGEVKNLRDWGIPLGRRFRALKLWFMLRSEGVEALQARLRRDLDNAQWLAGQIGAAAEWEVLAPVQLQTLCIRHRPAGLEGEALDAHTKGWAERLNASGDAYVTPATLDGRWMVRVSIGALPTEREHVEQLWARLQEVVKG

SEQ ID NO: 37 - protein, 500 aa, Catharanthus roseus
MGSIDSTNVAMSNSPVGEFKPLEAEEFRKQAHRMVDFIADYYKNVETYPVLSEVEPGYLRKRIPETAPYLPEPLDDIMKDIQKDIIPGMTNWMSPNFYAFFPATVSSAAFLGEMLSTALNSVGFTWVSSPAATELEMIVMDWLAQILKLPKSFMFSGTGGGVIQNTTSESILCTIIAARERALEKLGPDSIGKLVCYGSDQTHTMFPKTCKLAGIYPNNIRLIPTTVETDFGISPQVLRKMVEDDVAAGYVPLFLCATLGTTSTTATDPVDSLSEIANEFGIWIHVDAAYAGSACICPEFRHYLDGIERVDSLSLSPHKWLLAYLDCTCLWVKQPHLLLRALTTNPEYLKNKQSDLDKVVDFKNWQIATGRKFRSLKLWLILRSYGVVNLQSHIRSDVAMGKMFEEWVRSDSRFEIVVPRNFSLVCFRLKPDVSSLHVEEVNKKLLDMLNSTGRVYMTHTIVGGIYMLRLAVGSSLTEEHHVRRVWDLIQKLTDDLLKEA

SEQ ID NO: 38 - protein, 191 aa, Chlamydomonas reinhardtii
MAEESLDASVQPLGSTVFFGPVQPEMLDRIHELEAASYPEDEAATYEKLKFRIENASNVFLVALSAEGDGEPKVVGFVCGTQTRASKLTHESMSTHDADGALLCIHSVVVDAALRRRGLATRMLRAYTAFVAATSPGLTGIRLLTKQNLIPLYEGAGFTLLGPSDVEHGADLWYECAMELEAEEEAEAAEA

SEQ ID NO: 39 - protein, 207 aa, Bos taurus
MSTPSIHCLKPSPLHLPSGIPGSPGRQRRHTLPANEFRCLTPEDAAGVFEIEREAFISVSGNCPLNLDEVRHFLTLCPELSLGWFVEGRLVAFIIGSLWDEERLTQESLTLHRPGGRTAHLHALAVHHSFRQQGKGSVLLWRYLQHAGGQPAVRRAVLMCEDALVPFYQRFGFHPAGPCAVVVGSLTFTEMHCSLRGHAALRRNSDR

SEQ ID NO: 40 - protein, 207 aa, Bos taurus
MSTPSIHCLKPSPLHLPSGIPGSPGRQRRHTLPANEFRCLTPEDAAGVFEIEREPFISVSGNCPLNLDEVRHFLTLCPELSLGWFVEGRLVAFIIGSLWDEERLTQESLTLHRPGGRTAHLHALAVHHSFRQQGKGSVLLWRYLQHAGGQPAVRRAVLMCEDALVPFYQRFGFHPAGPCAVVVGSLTFTEMHCSLRGHAALRRNSDR

SEQ ID NO: 41 - protein, 205 aa, Gallus gallus
MPVLGAVPFLKPTPLQGPRNSPGRQRRHTLPASEFRCLSPEDAVSVFEIEREAFISVSGDCPLHLDEIRHFLTLCPELSLGWFEEGRLVAFIIGSLWDQDRLSQAALTLHNPRGTAVHIHVLAVHRTFRQQGKGSILMWRYLQYLRCLPCARRAVLMCEDFLVPFYEKCGFVAVGPCQVTVGTLAFTEMQHEVRGHAFMRRNSGC

SEQ ID NO: 42 - protein, 207 aa, Homo sapiens
MSTQSTHPLKPEAPRLPPGIPESPSCQRRHTLPASEFRCLTPEDAVSAFEIEREAFISVLGVCPLYLDEIRHFLTLCPELSLGWFEEGCLVAFIIGSLWDKERLMQESLTLHRSGGHIAHLHVLAVHRAFRQQGRGPILLWRYLHHLGSQPAVRRAALMCEDALVPFYERFSFHAVGPCAITVGSLTFMELHCSLRGHPFLRRNSGC

SEQ ID NO: 43 - protein, 205 aa, Mus musculus
MLNINSLKPEALHLPLGTSEFLGCQRRHTLPASEFRCLTPEDATSAFEIEREAFISVSGTCPLYLDEIRHFLTLCPELSLGWFEEGCLVAFIIGSLWDKERLTQESLTLHRPGGRTAHLHVLAVHRTFRQQGKGSVLLWRYLHHLGSQPAVRRAVLMCEDALVPFYEKFGFQAVGPCAITVGSLTFTELQCSLRCHAFLRRNSGC

SEQ ID NO: 44 - protein, 207 aa, Oryctolagus cuniculus
MSTLSTQPLKPKALHPPPGSPESPGHQRRHTLPASEFRCLTPEDAAGVFEIEREAFMSVSGSCPLYLDEIRHFLTLCPELSLGWFQEGRLVAFIIGSLWDKERLTQESLTLHRPGGRVAHLHVLAVHRACRQQGKGSVLLWRYLQHLGGQRAVRRAVLMCEDALVPFYERLGFRAVGPCAVTVGSLAFTELQCSVRGHACLRRKSGC

SEQ ID NO: 45 - protein, 207 aa, Ovis aries
MSTPSVHCLKPSPLHLPSGIPGSPGRQRRHTLPANEFRCLTPEDAAGVFEIEREAFISVSGNCPLNLDEVQHFLTLCPELSLGWFVEGRLVAFIIGSLWDEERLTQESLALHRPRGHSAHLHALAVHRSFRQQGKGSVLLWRYLHHVGAQPAVRRAVLMCEDALVPFYQRFGFHPAGPCAIVVGSLTFTEMHCSLRGHAALRRNSDR

SEQ ID NO: 46 - protein, 364 aa, Oryza sativa
MAQNVQENEQVMSTEDLLQAQIELYHHCLAFIKSMALRAATDLRIPDAIHCNGGAATLTDLAAHVGLHPTKLSHLRRLMRVLTLSGIFTVHDGDGEATYTLTRVSRLLLSDGVERTHGLSQMVRVFVNPVAVASQFSLHEWFTVEKAAAVSLFEVAHGCTRWEMIANDSKDGSMFNAGMVEDSSVAMDIILRKSSNVFRGINSLVDVGGGYGAVAAAVVRAFPDIKCTVLDLPHIVAKAPSNNNIQFVGGDLFEFIPAADVVLLKCILHCWQHDDCVKIMRRCKEAISARDAGGKVILIEVVVGIGSNETVPKEMQLLFDVFMMYTDGIEREEHEWKKIFLEAGFSDYKIIPVLGVRSIIEVYP

SEQ ID NO: 47 - protein, 345 aa, Homo sapiens
MGSSEDQAYRLLNDYANGFMVSQVLFAACELGVFDLLAEAPGPLDVAAVAAGVRASAHGTELLLDICVSLKLLKVETRGGKAFYRNTELSSDYLTTVSPTSQCSMLKYMGRTSYRCWGHLADAVREGRNQYLETFGVPAEELFTAIYRSEGERLQFMQALQEVWSVNGRSVLTAFDLSVFPLMCDLGGGAGALAKECMSLYPGCKITVFDIPEVVWTAKQHFSFQEEEQIDFQEGDFFKDPLPEADLYILARVLHDWADGKCSHLLERIYHTCKPGGGILVIESLLDEDRRGPLLTQLYSLNMLVQTEGQERTPTHYHMLLSSAGFRDFQFKKTGAIYDAILARK

SEQ ID NO: 48 - protein, 345 aa, Bos taurus
MCSQEGEGYSLLKEYANGFMVSQVLFAACELGVFELLAEALEPLDSAAVSSHLGSSPQGTELLLNTCVSLKLLQADVRGGKAVYANTELASTYLVRGSPRSQRDMLLYAGRTAYVCWRHLAEAVREGRNQYLKAFGIPSEELFSAIYRSEDERLQFMQGLQDVWRLEGATVLAAFDLSPFPLICDLGGGSGALAKACVSLYPGCRAIVFDIPGVVQIAKRHFSASEDERISFHEGDFFKDALPEADLYILARVLHDWTDAKCSHLLQRVYRACRTGGGILVIESLLDTDGRGPLTTLLYSLNMLVQTEGRERTPAEYRALLGPAGFRDVRCRRTGGTYDAVLARK

SEQ ID NO: 49 - protein, 432 aa, Rattus norwegicus
MAPGREGELDRDFRVLMSLAHGFMVSQVLFAALDLGIFDLAAQGPVAAEAVAQTGGWSPRGTQLLMDACTRLGLLRGAGDGSYTNSALSSTFLVSGSPQSQRCMLLYLAGTTYGCWAHLAAGVREGRNQYSRAVGISAEDPFSAIYRSEPERLLFMRGLQETWSLCGGRVLTAFDLSRFRVICDLGGGSGALAQEAARLYPGSSVCVFDLPDVIAAARTHFLSPGARPSVRFVAGDFFRSRLPRADLFILARVLHDWADGACVELLGRLHRACRPGGALLLVEAVLAKGGAGPLRSLLLSLNMMLQAEGWERQASDYRNLATRAGFPRLQLRRPGGPYHAMLARRGPRPGIITGVGSNTTGTGSFVTGIRRDVPGARSDAAGTGSGTGNTGSGIMLQGETLESEVSAPQAGSDVGGAGNEPRSGTLKQGDWK

SEQ ID NO: 50 - protein, 346 aa, Gallus gallus
MDSTEDLDYPQIIFQYSNGFLVSKVMFTACELGVFDLLLQSGRPLSLDVIAARLGTSIMGMERLLDACVGLKLLAVELRREGAFYRNTEISNIYLTKSSPKSQYHIMMYYSNTVYLCWHYLTDAVREGRNQYERAFGISSKDLFGARYRSEEEMLKFLAGQNSIWSICGRDVLTAFDLSPFTQIYDLGGGGGALAQECVFLYPNCTVTIYDLPKVVQVAKERLVPPEERRIAFHEGDFFKDSIPEADLYILSKILHDWDDKKCRQLLAEVYKACRPGGGVLLVESLLSEDRSGPVETQLYSLNMLVQTEGKERTAVEYSELLGAAGFREVQVRRTGKLYDAVLGRK

SEQ ID NO: 51 - protein, 345 aa, Macaca mulatta
MGSSGDDGYRLLNEYTNGFMVSQVLFAACELGVFDLLAEAPGPLDVAAVAAGVEASSHGTELLLDTCVSLKLLKVETRAGKAFYQNTELSSAYLTRVSPTSQCNLLKYMGRTSYGCWGHLADAVREGKNQYLQTFGVPAEDLFKAIYRSEGERLQFMQALQEVWSVNGRSVLTAFDLSGFPLMCDLGGGPGALAKECLSLYPGCKVTVFDVPEVVRTAKQHFSFPEEEEIHLQEGDFFKDPLPEADLYILARILHDWADGKCSHLLERVYHTCKPGGGILVIESLLDEDRRGPLLTQLYSLNMLVQTEGQERTPTHYHMLLSSAGFRDFQFKKTGAIYDAILVRK

SEQ ID NO: 52 - protein, 298 aa, Escherichia coli
MLEKSLATLFALLILATLINRFLLWRLPERKGGEVTLRIRTWWGIVICFSMVISGPRWMTLTFFALISFLALKEYCTLISVHFPRWLYWGIPLNYLLIGFNCFELFLLFIPLAGFLILATGQVLVGDPSGFLHTVSAIFWGWIMTVFALSHAAWLLMLPTTNIQGGALLVLFLLALTESNDIAQYLWGKSCGRRKVVPKVSPGKTLEGLMGGVITIMIASLIIGPLLTPLNTLQALLAGLLIGISGFCGDVVMSAIKRDIGVKDSGKLLPGHGGLLDRIDSLIFTAPVFFYFIRYCCY

SEQ ID NO: 53 - DNA, 71 bp, Artificial
  Ptrc promoter and 5' coding sequence
tgacaattaatcatccggctcgtataatgtgtggaattgtgagcggataacaatttcacacaggagtaaaa

SEQ ID NO: 54 - protein, 528 aa, Homo sapiens
MPTPDATTPQAKGFRRAVSELDAKQAEAIMVRGQGAPGPSLTGSPWPGTAAPAASYTPTPRSPRFIGRRQSLIEDARKEREAAVAAAAAAVPSEPGDPLEAVAFEEKEGKAVLNLLFSPRATKPSALSRAVKVFETFEAKIHHLETRPAQRPRAGGPHLEYFVRLEVRRGDLAALLSGVRQVSEDVRSPAGPKVPWFPRKVSELDKCHHLVTKFDPDLDLDHPGFSDQVYRQRRKLIAEIAFQYRHGDPIPRVEYTAEEIATWKEVYTTLKGLYATHACGEHLEAFALLERFSGYREDNIPQLEDVSRFLKERTGFQLRPVAGLLSARDFLASLAFRVFQCTQYIRHASSPMHSPEPDCCHELLGHVPMLADRTFAQFSQDIGLASLGASDEEIEKLSTLYWFTVEFGLCKQNGEVKAYGAGLLSSYGELLHCLSEEPEIRAFDPEAAAVQPYQDQTYQSVYFVSESFSDAKDKLRSYASRIQRPFSVKFDPYTLAIDVLDSPQAVRRSLEGVQDELDTLAHALSAIG

SEQ ID NO: 55 - protein, 498 aa, Mus musculus
MPTPSASSPQPKGFRRAVSEQDTKQAEAVTSPRFIGRRQSLIEDARKEREAAAAAAAAAVASAEPGNPLEAVVFEERDGNAVLNLLFSLRGTKPSSLSRALKVFETFEAKIHHLETRPAQRPLAGSPHLEYFVRFEVPSGDLAALLSSVRRVSDDVRSAREDKVPWFPRKVSELDKCHHLVTKFDPDLDLDHPGFSDQAYRQRRKLIAEIAFQYKQGEPIPHVEYTKEEIATWKEVYATLKGLYATHACREHLEAFQLLERYCGYREDSIPQLEDVSHFLKERTGFQLRPVAGLLSARDFLASLAFRVFQCTQYIRHASSPMHSPEPDCCHELLGHVPMLADRTFAQFSQDIGLASLGASDEEIEKLSTVYWFTVEFGLCKQNGELKAYGAGLLSSYGELLHSLSEEPEVRAFDPDTAAVQPYQDQTYQPVYFVSESFSDAKDKLRNYASRIQRPFSVKFDPYTLAIDVLDSPHTIRRSLEGVQDELHTLTQALSAIS

SEQ ID NO: 56 - protein, 491 aa, Bos taurus
MPTPNAASPQAKGFRRAVSELDAKQAEAIMSPRFVGRRQSLIQDARKEREKAEAAASSSESAEAAAWLERDGEAVLTLLFALPPTRPPALTRAIKVFETFEAHLHHLETRPAQPLRAGSPPLECFVRCEVPGPVVPALLSALRRVAEDVRAAGESKVLWFPRKVSELDKCHHLVTKFDPDLDLDHPGFSDQAYRQRRKLIAEIAFQYKQGDPIPHVEYTAEETATWKEVYSTLRGLYPTHACREHLEAFELLERFCGYREDRIPQLEDVSRFLKERTGFQLRPAAGLLSARDFLASLAFRVFQCTQYIRHASSPMHSPEPECCHELLGHVPMLADRTFAQFSQDIGLASLGVSDEEIEKLSTLYWFTVEFGLCKQNGEVKAYGAGLLSSYGELLHSLSEEPEIRAFDPDAAAVQPYQDQTYQPVYFVSESFSDAKDKLRSYASRIQRPFSVKFDPYTLAIDVLDSPHAIRHALDGVQDEMQALAHALNAIS

SEQ ID NO: 57 - protein, 491 aa, Gallus gallus
MPTPNISTSAAKGFRRAVSELDSKQAEAIMSPRFIGRRQSLIEDARKEREAAAAATDAAESTETIVFEEKDGRAMLNLFFMLKGAKTSPLSRALKVFETFEAKIHHLETRLSRKPREGTAELEYFVRCEVHSSDLNTFISSIKRVAEDVRTTKEDKFHWFPRKICELDKCHHLVTKFDPDLDLDHPGYSDQVYRQRRKSIAEIAFHYKHGDPIPRVEYTAEETATWKEVYSTLKSLYPTHACKEYLEAFNLLEKFCGYNENNIPQLEEVSRFLKERTGFQLRPVAGLLSARDFLASLAFRVFQCTQYIRHASSPMHSPEPDCCHELLGHVPMLADKTFAQFSQDIGLASLGATDEEIEKLATLYWFTVEFGLCRQNGIVKAYGAGLLSSYGELIHSLSDEPEVRDFDPDAAAVQPYQDQNYQPVYFVSESFSDAKNKLRNYAAHIKRPFSVKYEPYTHSIELLDSPQTICHSLESVRDELHSLINALNVIS

SEQ ID NO: 58 - protein, 297 aa, Chromobacterium violaceum
MNDRADFVVPDITTRKNVGLSHDANDFTLPQPLDRYSAEDHATWATLYQRQCKLLPGRACDEFMEGLERLEVDADRVPDFNKLNQKLMAATGWKIVAVPGLIPDDVFFEHLANRRFPVTWWLREPHQLDYLQEPDVFHDLFGHVPLLINPVFADYLEAYGKGGVKAKALGALPMLARLYWYTVEFGLINTPAGMRIYGAGILSSKSESIYCLDSASPNRVGFDLMRIMNTRYRIDTFQKTYFVIDSFKQLFDATAPDFAPLYLQLADAQPWGAGDVAPDDLVLNAGDRQGWADTEDV

SEQ ID NO: 59 - protein, 272 aa, Xanthomonas campestris
MVEQPWDGYSADDHATWGTLYRRQRELLVGRACEEFLQAQDAMGMGQTHIPRFDALNRVLQAATGWTLVGVQGLLPELDFFDHLANRRFPVTWWIRRPDQIDYIAEPDLFHDLFGHVPLLMNPLFADFMQAYGRGGVKAHGIGPDALQNLTRLYWYTVEFGLIDTPQGLRIYGAGIVSSKGESLYSLESPAPNRIGFDLQRIMRTRYRIDSFQKTYFVIDSFAQLMEATAPDFTPIYAELAQQPQVPAGDVLPGDRVIQRGSGEGWSRDGDV

SEQ ID NO: 60 - protein, 262 aa, Pseudomonas aeruginosa
MKTTQYVARQPDDNGFIHYPETEHQVWNTLITRQLKVIEGRACQEYLDGIEQLGLPHERIPQLDEINRVLQATTGWRVARVPALIPFQTFFELLASQQFPVATFIRTPEELDYLQEPDIFHEIFGHCPLLTNPWFAEFTHTYGKLGLKASKEERVFLARLYWMTIEFGLVETDQGKRIYGGGILSSPKETVYSLSDEPLHQAFNPLEAMRTPYRIDILQPLYFVLPDLKRLFQLAQEDIMALVHEAMRLGLHAPLFPPKQAA

SEQ ID NO: 61 - protein, 262 aa, Pseudomonas putida
MKQTQYVAREPDAHGFIDYPQQEHAVWNTLITRQLKVIEGRACQEYLDGIDQLKLPHDRIPQLGEVNKVLGATTGWQVARVPALIPFQTFFELLASKRFPVATFIRTPEELDYLQEPDIFHEIFGHCPLLTNPWFAEFTHTYGKLGLAATKEQRVYLARLYWMTIEFGLMETPQGRKIYGGGILSSPKETVYSLSGEPEHQAFDPIEAMRTPYRIDILQPLYFVLPNMKRLFDLAHEDIMGMVHKAMQLGLHAPKFPPKVAA

SEQ ID NO: 62 - protein, 452 aa, Homo sapiens
MSTAVLENPGLGRKLSDFGQETSYIEDNCNQNGAISLIFSLKEEVGALAKVLRLFEENDVNLTHIESRPSRLKKDEYEFFTHLDKRSLPALTNIIKILRHDIGATVHELSRDKKKDTVPWFPRTIQELDRFANQILSYGAELDADHPGFKDPVYRARRKQFADIAYNYRHGQPIPRVEYMEEEKKTWGTVFKTLKSLYKTHACYEYNHIFPLLEKYCGFHEDNIPQLEDVSQFLQTCTGFRLRPVAGLLSSRDFLGGLAFRVFHCTQYIRHGSKPMYTPEPDICHELLGHVPLFSDRSFAQFSQEIGLASLGAPDEYIEKLATIYWFTVEFGLCKQGDSIKAYGAGLLSSFGELQYCLSEKPKLLPLELEKTAIQNYTVTEFQPLYYVAESFNDAKEKVRNFAATIPRPFSVRYDPYTQRIEVLDNTQQLKILADSINSEIGILCSALQKIK

SEQ ID NO: 63 - protein, 453 aa, Mus musculus
MAAVVLENGVLSRKLSDFGQETSYIEDNSNQNGAVSLIFSLKEEVGALAKVLRLFEENEINLTHIESRPSRLNKDEYEFFTYLDKRSKPVLGSIIKSLRNDIGATVHELSRDKEKNTVPWFPRTIQELDRFANQILSYGAELDADHPGFKDPVYRARRKQFADIAYNYRHGQPIPRVEYTEEERKTWGTVFRTLKALYKTHACYEHNHIFPLLEKYCGFREDNIPQLEDVSQFLQTCTGFRLRPVAGLLSSRDFLGGLAFRVFHCTQYIRHGSKPMYTPEPDICHELLGHVPLFSDRSFAQFSQEIGLASLGAPDEYIEKLATIYWFTVEFGLCKEGDSIKAYGAGLLSSFGELQYCLSDKPKLLPLELEKTACQEYTVTEFQPLYYVAESFNDAKEKVRTFAATIPRPFSVRYDPYTQRVEVLDNTQQLKILADSINSEVGILCHALQKIKS

SEQ ID NO: 64 - protein, 279 aa, Streptomyces coeruleorubidus
MQGPHAQMTDAAYEIRRSEIAALSTDLAPEDPIPVVEYTEWEHEVWRTVCVDLTARHRTDAAAEYLESAEQLAVPLDHVPQLRDVSGRLGSISGFTFQSAPALVPLREFCGGLANSVFHSTQYLRHPRSPFYTEDPDLLHDLVGHGNVLASDRFARLYRLAGNAAARVHSTEALQFIGKVFWFTLECGVVRERGERKAYGATLVSSYGELDHFRSADFRPLDIKSLADVEYDISTYQPILFEADSMDEVEDTVGSFWDTCDDDSIAALLGGTSRSVTPH